European Patent Application EP 4 261 224 A1, published October 18, 2023. Title: CD73 ANTIGEN-BINDING PROTEIN AND APPLICATION THEREOF. Applicant: SHANGHAI HUAOTA BIOPHARMACEUTICAL CO.,LTD.;HUABO BIOPHARM (SHANGHAI) CO.,LTD. The sequence listing filed with the application follows.

SEQUENCE LISTING (47 sequences)

SEQ ID NO: 1 - protein, 8 aa, Artificial Sequence
  900581 HCDR1
GFTFSKYA

SEQ ID NO: 2 - protein, 8 aa, Artificial Sequence
  900581 HCDR2
ISSGGGYI

SEQ ID NO: 3 - protein, 18 aa, Artificial Sequence
  900581 HCDR3
ARAIYYYGSSYNYYAMDY

SEQ ID NO: 4 - protein, 6 aa, Artificial Sequence
  900581 LCDR1
QDVGTA

SEQ ID NO: 5 - protein, 3 aa, Artificial Sequence
  900581 LCDR2
WAS

SEQ ID NO: 6 - protein, 9 aa, Artificial Sequence
  900581 LCDR3
QQYSSYPLT

SEQ ID NO: 7 - protein, 25 aa, Artificial Sequence
  900581 H-FR1
EVQLVESGGGLVKPGGSLKLSCAAS

SEQ ID NO: 8 - protein, 17 aa, Artificial Sequence
  900581 H-FR2
MSWVRQSPEKRLEWVAE

SEQ ID NO: 9 - protein, 38 aa, Artificial Sequence
  900581 H-FR3
NYPDTVTGRFTISRDNAKNTLYLEMSSLRSGDTAMYYC

SEQ ID NO: 10 - protein, 11 aa, Artificial Sequence
  900581 H-FR4
WGQGTSVTVSS

SEQ ID NO: 11 - protein, 26 aa, Artificial Sequence
  900581 L-FR1
DIVMTQSHKFMSTSVGDRVSITCKAS

SEQ ID NO: 12 - protein, 17 aa, Artificial Sequence
  900581 L-FR2
EAWYQQKPGQSPKLLIY

SEQ ID NO: 13 - protein, 36 aa, Artificial Sequence
  900581 L-FR3
TRHTGVPDRFTGSGSGTDFTLTIGNVQSEDLADYFC

SEQ ID NO: 14 - protein, 10 aa, Artificial Sequence
  900581 L-FR4
FGGGTKLEIK

SEQ ID NO: 15 - protein, 25 aa, Artificial Sequence
  900694 H-FR1
EVQLVESGGGLVKPGGSLRLSCAAS

SEQ ID NO: 16 - protein, 17 aa, Artificial Sequence
  H-FR2 of 900694 900695 900697
MSWVRQAPGKGLEWVAE

SEQ ID NO: 17 - protein, 38 aa, Artificial Sequence
  900694 H-FR3
NYPDTVTGRFTISRDNAKNSLYLQMNSLRAEDTAVYYC

SEQ ID NO: 18 - protein, 11 aa, Artificial Sequence
  H-FR4 of 900694 900695 900696 900697 900698
WGQGTTVTVSS

SEQ ID NO: 19 - protein, 25 aa, Artificial Sequence
  H-FR1 of 900695 900697 90069 900698
QVQLVESGGGLVKPGGSLRLSCAAS

SEQ ID NO: 20 - protein, 38 aa, Artificial Sequence
  H-FR3 of 900695 900697
NYADSVTGRFTISRDNAKNSLYLQMNSLRAEDTAVYYC

SEQ ID NO: 21 - protein, 17 aa, Artificial Sequence
  H-FR2 of 900696 900698
MSWIRQAPGKGLEWVAE

SEQ ID NO: 22 - protein, 38 aa, Artificial Sequence
  H-FR3 of 900696 900698
NYADSVKGRFTISRDNAKNSLYLQMNSLRAEDTAVYYC

SEQ ID NO: 23 - protein, 26 aa, Artificial Sequence [sequence omitted]

SEQ ID NO: 24 - protein, 17 aa, Artificial Sequence
  L-FR2 of 900694 900695 900696 900697 900698
EAWYQQKPGKAPKLLIY

SEQ ID NO: 25 - protein, 36 aa, Artificial Sequence
  900694 L-FR3
TRHTGVPDRFSGSGSGTDFTLTISSLQPEDFATYYC

SEQ ID NO: 26 - protein, 10 aa, Artificial Sequence
  L-FR4 900694 900695 900696 900697 900698
FGQGTKLEIK

SEQ ID NO: 27 - protein, 36 aa, Artificial Sequence
  L-FR3 of 900695 900698
TRHTGVPSRFSGSGSGTDFTLTISSLQPEDFATYYC

SEQ ID NO: 28 - protein, 36 aa, Artificial Sequence
  L-FR3 of 900696 900697
TLQSGVPSRFSGSGSGTDFTLTISSLQPEDFATYYC

SEQ ID NO: 29 - protein, 125 aa, Artificial Sequence
  900581 VH
EVQLVESGGGLVKPGGSLKLSCAASGFTFSKYAMSWVRQSPEKRLEWVAEISSGGGYINYPDTVTGRFTISRDNAKNTLYLEMSSLRSGDTAMYYCARAIYYYGSSYNYYAMDYWGQGTSVTVSS

SEQ ID NO: 30 - protein, 107 aa, Artificial Sequence
  900581 VL
DIVMTQSHKFMSTSVGDRVSITCKASQDVGTAEAWYQQKPGQSPKLLIYWASTRHTGVPDRFTGSGSGTDFTLTIGNVQSEDLADYFCQQYSSYPLTFGGGTKLEIK

SEQ ID NO: 31 - protein, 125 aa, Artificial Sequence
  900694 VH
EVQLVESGGGLVKPGGSLRLSCAASGFTFSKYAMSWVRQAPGKGLEWVAEISSGGGYINYPDTVTGRFTISRDNAKNSLYLQMNSLRAEDTAVYYCARAIYYYGSSYNYYAMDYWGQGTTVTVSS

SEQ ID NO: 32 - protein, 107 aa, Artificial Sequence
  900694 VL
DIQMTQSPSSLSASVGDRVTITCRASQDVGTAEAWYQQKPGKAPKLLIYWASTRHTGVPDRFSGSGSGTDFTLTISSLQPEDFATYYCQQYSSYPLTFGQGTKLEIK

SEQ ID NO: 33 - protein, 125 aa, Artificial Sequence
  VH of 900695 900697
QVQLVESGGGLVKPGGSLRLSCAASGFTFSKYAMSWVRQAPGKGLEWVAEISSGGGYINYADSVTGRFTISRDNAKNSLYLQMNSLRAEDTAVYYCARAIYYYGSSYNYYAMDYWGQGTTVTVSS

SEQ ID NO: 34 - protein, 107 aa, Artificial Sequence
  VL of 90069 900698
DIQMTQSPSSLSASVGDRVTITCRASQDVGTAEAWYQQKPGKAPKLLIYWASTRHTGVPSRFSGSGSGTDFTLTISSLQPEDFATYYCQQYSSYPLTFGQGTKLEIK

SEQ ID NO: 35 - protein, 125 aa, Artificial Sequence
  VH of 900696 900698
QVQLVESGGGLVKPGGSLRLSCAASGFTFSKYAMSWIRQAPGKGLEWVAEISSGGGYINYADSVKGRFTISRDNAKNSLYLQMNSLRAEDTAVYYCARAIYYYGSSYNYYAMDYWGQGTTVTVSS

SEQ ID NO: 36 - protein, 107 aa, Artificial Sequence
  VL of 900696 900697
DIQMTQSPSSLSASVGDRVTITCRASQDVGTAEAWYQQKPGKAPKLLIYWASTLQSGVPSRFSGSGSGTDFTLTISSLQPEDFATYYCQQYSSYPLTFGQGTKLEIK

SEQ ID NO: 37 - protein, 15 aa, Artificial Sequence
  amino acids 143 to 157 a of CD73
NIKAKGPLASQISGL

SEQ ID NO: 38 - protein, 14 aa, Artificial Sequence
  amino acids 178-191 of CD73
SKETPFLSNPGTNL

SEQ ID NO: 39 - protein, 6 aa, Artificial Sequence
  amino acids of 381-386 of CD73
WNHVSM

SEQ ID NO: 40 - protein, 574 aa, Artificial Sequence
  CD73 full length sequence
MCPRAARAPATLLLALGAVLWPAAGAWELTILHTNDVHSRLEQTSEDSSKCVNASRCMGGVARLFTKVQQIRRAEPNVLLLDAGDQYQGTIWFTVYKGAEVAHFMNALRYDAMALGNHEFDNGVEGLIEPLLKEAKFPILSANIKAKGPLASQISGLYLPYKVLPVGDEVVGIVGYTSKETPFLSNPGTNLVFEDEITALQPEVDKLKTLNVNKIIALGHSGFEMDKLIAQKVRGVDVVVGGHSNTFLYTGNPPSKEVPAGKYPFIVTSDDGRKVPVVQAYAFGKYLGYLKIEFDERGNVISSHGNPILLNSSIPEDPSIKADINKWRIKLDNYSTQELGKTIVYLDGSSQSCRFRECNMGNLICDAMINNNLRHTDEMFWNHVSMCILNGGGIRSPIDERNNGTITWENLAAVLPFGGTFDLVQLKGSTLKKAFEHSVHRYGQSTGEFLQVGGIHVVYDLSRKPGDRVVKLDVLCTKCRVPSYDPLKMDEVYKVILPNFLANGGDGFQMIKDELLRHDSGDQDINVVSTYISKMKVIYPAVEGRIKFSTGSHCHGSFSLIFLSLWAVIFVLYQ

SEQ ID NO: 41 - protein, 122 aa, Artificial Sequence
  900565 VH
QAYLQQSGAELVRPGASVKMSCKASGYTFTSYNMHWVKQTPRQGLEWIGAIYPGNGDTSYNQKFKGKATLNVDKSSSTAYMQLSSLTSEDSAVYFCARWGYGSNYAWYFDIWGTGTTVTVSS

SEQ ID NO: 42 - protein, 107 aa, Artificial Sequence
  900565 VL
DIQMTQSPASLSASVGETVTITCRTSGNIHNYLVWYQQKQGKSPQLLVFNAKTLADGVPSRFSGSGSGTQYSLKINSLQPEDFGSYYCQHFWSTPFTFGSGTKLEIK

SEQ ID NO: 43 - protein, 450 aa, Artificial Sequence
  900201 HC
QIQLVQSGPELKKPGETVKISCKTSGYTFTNYGMNWVKQAPGKGLKWVGWINTYTGEPKYADDFKGRFAFSVETSASTAYLQINNLKNEDTATYFCARGIYDGYHWYFDVWGAGTTVTVSSASTKGPSVFPLAPSSKSTSGGTAALGCLVKDYFPEPVTVSWNSGALTSGVHTFPAVLQSSGLYSLSSVVTVPSSSLGTQTYICNVNHKPSNTKVDKRVEPKSCDKTHTCPPCPAPELLGGPSVFLFPPKPKDTLMISRTPEVTCVVVDVSHEDPEVKFNWYVDGVEVHNAKTKPREEQYNSTYRVVSVLTVLHQDWLNGKEYKCKVSNKALPAPIEKTISKAKGQPREPQVYTLPPSREEMTKNQVSLTCLVKGFYPSDIAVEWESNGQPENNYKTTPPVLDSDGSFFLYSKLTVDKSRWQQGNVFSCSVMHEALHNHYTQKSLSLSPG

SEQ ID NO: 44 - protein, 219 aa, Artificial Sequence
  900201 LC
DVVMTQTPLSLPVSLGDQASISCRSSQSLVHSIGNTYLHWYLQKPGQSPKLLIYKVSNRFSGVPDRFSGSGSGTDFTLKITRVEAEDLGVYFCSQSTHVPFTFGSGTKLEIKRTVAAPSVFIFPPSDEQLKSGTASVVCLLNNFYPREAKVQWKVDNALQSGNSQESVTEQDSKDSTYSLSSTLTLSKADYEKHKVYACEVTHQGLSSPVTKSFNRGEC

SEQ ID NO: 45 - protein, 447 aa, Artificial Sequence
  Oleclumab HC
EVQLLESGGGLVQPGGSLRLSCAASGFTFSSYAYSWVRQAPGKGLEWVSAISGSGGRTYYADSVKGRFTISRDNSKNTLYLQMNSLRAEDTAVYYCARLGYGRVDEWGRGTLVTVSSASTKGPSVFPLAPSSKSTSGGTAALGCLVKDYFPEPVTVSWNSGALTSGVHTFPAVLQSSGLYSLSSVVTVPSSSLGTQTYICNVNHKPSNTKVDKRVEPKSCDKTHTCPPCPAPEFEGGPSVFLFPPKPKDTLMISRTPEVTCVVVDVSHEDPEVKFNWYVDGVEVHNAKTKPREEQYNSTYRVVSVLTVLHQDWLNGKEYKCKVSNKALPASIEKTISKAKGQPREPQVYTLPPSREEMTKNQVSLTCLVKGFYPSDIAVEWESNGQPENNYKTTPPVLDSDGSFFLYSKLTVDKSRWQQGNVFSCSVMHEALHNHYTQKSLSLSPGK

SEQ ID NO: 46 - protein, 216 aa, Artificial Sequence
  Oleclumab LC
QSVLTQPPSASGTPGQRVTISCSGSLSNIGRNPVNWYQQLPGTAPKLLIYLDNLRLSGVPDRFSGSKSGTSASLAISGLQSEDEADYYCATWDDSHPGWTFGGGTKLTVLGQPKAAPSVTLFPPSSEELQANKATLVCLISDFYPGAVTVAWKADSSPVKAGVETTTPSKQSNNKYAASSYLSLTPEQWKSHRSYSCQVTHEGSTVEKTVAPTECS

SEQ ID NO: 47 - protein, 450 aa, Artificial Sequence
  900543 HC
QIQLVQSGPELKKPGETVKISCKTSGYTFTNYGMNWVKQAPGKGLKWVGWINTYTGEPKYADDFKGRFAFSVETSASTAYLQINNLKNEDTATYFCARGIYDGYHWYFDVWGAGTTVTVSSASTKGPSVFPLAPSSKSTSGGTAALGCLVKDYFPEPVTVSWNSGALTSGVHTFPAVLQSSGLYSLSSVVTVPSSSLGTQTYICNVNHKPSNTKVDKRVEPKSCDKTHTCPPCPAPEAAGGPSVFLFPPKPKDTLMISRTPEVTCVVVDVSHEDPEVKFNWYVDGVEVHNAKTKPREEQYNSTYRVVSVLTVLHQDWLNGKEYKCKVSNKALPAPIEKTISKAKGQPREPQVYTLPPSREEMTKNQVSLTCLVKGFYPSDIAVEWESNGQPENNYKTTPPVLDSDGSFFLYSKLTVDKSRWQQGNVFSCSVMHEALHNHYTQKSLSLSPG